European Patent Application EP 4 309 669 A1, published January 24, 2024. Title: UNIVERSAL CHIMERIC ANTIGEN RECEPTOR T-CELL AND APPLICATION THEREOF. Applicant: SHANGHAI IASO BIOTECHNOLOGY CO., LTD. The sequence listing filed with the application follows.

SEQUENCE LISTING (82 sequences)

SEQ ID NO: 1 - DNA, 21 bp, Artificial
  LCK-sgRNA12-21nt   target DNA sequence
tctacatcatcactgaataca

SEQ ID NO: 2 - DNA, 20 bp, Artificial
  LCK-sgRNA12-20nt   target DNA sequence
ctacatcatcactgaataca

SEQ ID NO: 3 - DNA, 19 bp, Artificial
  LCK-sgRNA12-19nt   target DNA sequence
tacatcatcactgaataca

SEQ ID NO: 4 - DNA, 18 bp, Artificial
  LCK-sgRNA12-18nt  target DNA sequence
acatcatcactgaataca

SEQ ID NO: 5 - DNA, 21 bp, Artificial
  LCK-sgRNA16-21nt   target DNA sequence
catcactgaatacatggagaa

SEQ ID NO: 6 - DNA, 20 bp, Artificial
  LCK-sgRNA16-20nt   target DNA sequence
atcactgaatacatggagaa

SEQ ID NO: 7 - DNA, 19 bp, Artificial
  LCK-sgRNA16-19nt   target DNA sequence
tcactgaatacatggagaa

SEQ ID NO: 8 - DNA, 18 bp, Artificial
  LCK-sgRNA16-18nt   target DNA sequence
cactgaatacatggagaa

SEQ ID NO: 9 - protein, 509 aa, Artificial
  LCK-T316I mutant protein sequence
MGCGCSSHPEDDWMENIDVCENCHYPIVPLDGKGTLLIRNGSEVRDPLVTYEGSNPPASPLQDNLVIALHSYEPSHDGDLGFEKGEQLRILEQSGEWWKAQSLTTGQEGFIPFNFVAKANSLEPEPWFFKNLSRKDAERQLLAPGNTHGSFLIRESESTAGSFSLSVRDFDQNQGEVVKHYKIRNLDNGGFYISPRITFPGLHELVRHYTNASDGLCTRLSRPCQTQKPQKPWWEDEWEVPRETLKLVERLGAGQFGEVWMGYYNGHTKVAVKSLKQGSMSPDAFLAEANLMKQLQHQRLVRLYAVVTQEPIYIIIEYMENGSLVDFLKTPSGIKLTINKLLDMAAQIAEGMAFIEERNYIHRDLRAANILVSDTLSCKIADFGLARLIEDNEYTAREGAKFPIKWTAPEAINYGTFTIKSDVWSFGILLTEIVTHGRIPYPGMTNPEVIQNLERGYRMVRPDNCPEELYQLMRLCWKERPEDRPTFDYLRSVLEDFFTATEGQYQPQP

SEQ ID NO: 10 - protein, 509 aa, Artificial
  LCK-T316A mutant protein sequence
MGCGCSSHPEDDWMENIDVCENCHYPIVPLDGKGTLLIRNGSEVRDPLVTYEGSNPPASPLQDNLVIALHSYEPSHDGDLGFEKGEQLRILEQSGEWWKAQSLTTGQEGFIPFNFVAKANSLEPEPWFFKNLSRKDAERQLLAPGNTHGSFLIRESESTAGSFSLSVRDFDQNQGEVVKHYKIRNLDNGGFYISPRITFPGLHELVRHYTNASDGLCTRLSRPCQTQKPQKPWWEDEWEVPRETLKLVERLGAGQFGEVWMGYYNGHTKVAVKSLKQGSMSPDAFLAEANLMKQLQHQRLVRLYAVVTQEPIYIIAEYMENGSLVDFLKTPSGIKLTINKLLDMAAQIAEGMAFIEERNYIHRDLRAANILVSDTLSCKIADFGLARLIEDNEYTAREGAKFPIKWTAPEAINYGTFTIKSDVWSFGILLTEIVTHGRIPYPGMTNPEVIQNLERGYRMVRPDNCPEELYQLMRLCWKERPEDRPTFDYLRSVLEDFFTATEGQYQPQP

SEQ ID NO: 11 - protein, 509 aa, Artificial
  LCK-T316M mutant protein sequence
MGCGCSSHPEDDWMENIDVCENCHYPIVPLDGKGTLLIRNGSEVRDPLVTYEGSNPPASPLQDNLVIALHSYEPSHDGDLGFEKGEQLRILEQSGEWWKAQSLTTGQEGFIPFNFVAKANSLEPEPWFFKNLSRKDAERQLLAPGNTHGSFLIRESESTAGSFSLSVRDFDQNQGEVVKHYKIRNLDNGGFYISPRITFPGLHELVRHYTNASDGLCTRLSRPCQTQKPQKPWWEDEWEVPRETLKLVERLGAGQFGEVWMGYYNGHTKVAVKSLKQGSMSPDAFLAEANLMKQLQHQRLVRLYAVVTQEPIYIIMEYMENGSLVDFLKTPSGIKLTINKLLDMAAQIAEGMAFIEERNYIHRDLRAANILVSDTLSCKIADFGLARLIEDNEYTAREGAKFPIKWTAPEAINYGTFTIKSDVWSFGILLTEIVTHGRIPYPGMTNPEVIQNLERGYRMVRPDNCPEELYQLMRLCWKERPEDRPTFDYLRSVLEDFFTATEGQYQPQP

SEQ ID NO: 12 - DNA, 22 bp, Artificial
  LCK-saCas9-sgRNA1 target DNA sequence
ctacatcatcactgaatacatg

SEQ ID NO: 13 - DNA, 22 bp, Artificial
  LCK-saCas9-sgRNA2 target DNA sequence
atcactgaatacatggagaatg

SEQ ID NO: 14 - DNA, 20 bp, Artificial
  LCK-sgRNA1    target DNA sequence
gctacccgagtcggctacca

SEQ ID NO: 15 - DNA, 20 bp, Artificial
  LCK-sgRNA11    target DNA sequence
gctctacgctgtggtcaccc

SEQ ID NO: 16 - DNA, 20 bp, Artificial
  LCK-sgRNA8    target DNA sequence
gtattcagtgatgatgtaga

SEQ ID NO: 17 - DNA, 20 bp, Artificial
  LCK-sgRNA9    target DNA sequence
tattcagtgatgatgtagat

SEQ ID NO: 18 - DNA, 20 bp, Artificial
  LCK-sgRNA12    target DNA sequence
ctacatcatcactgaataca

SEQ ID NO: 19 - DNA, 135 bp, Artificial
  ssDNA-T316I-for-sgRNA8   DNA sequence as repair template
acgccttcctggccgaggccaacctcatgaagcagctgcaacaccagcggctggttcggctctacgctgtggtcacccaggagcccatctacatcatcattgaatacatggagaatggtgggtgctacccgagtc

SEQ ID NO: 20 - DNA, 135 bp, Artificial
  ssDNA-T316I-for-sgRNA9  DNA sequence as repair template
gacgccttcctggccgaggccaacctcatgaagcagctgcaacaccagcggctggttcggctctacgctgtggtcacccaggagcccatctacatcatcattgaatacatggagaatggtgggtgctacccgagt

SEQ ID NO: 21 - DNA, 135 bp, Artificial
  ssDNA-T316I-for-sgRNA12  DNA sequence as repair template
aaaaggtgtatttccaccctctggcagggacagcagggagagcagtatcccctggtagccgactcgggtagcacccaccattctccatgtattcaatgatgatgtagatgggctcctgggtgaccacagcgtaga

SEQ ID NO: 22 - DNA, 135 bp, Artificial
  ssDNA-T316M-for-sgRNA8  DNA sequence as repair template
acgccttcctggccgaggccaacctcatgaagcagctgcaacaccagcggctggttcggctctacgctgtggtcacccaggagcccatctacatcatcatggaatacatggagaatggtgggtgctacccgagtc

SEQ ID NO: 23 - DNA, 135 bp, Artificial
  ssDNA-T316M-for-sgRNA9  DNA sequence as repair template
gacgccttcctggccgaggccaacctcatgaagcagctgcaacaccagcggctggttcggctctacgctgtggtcacccaggagcccatctacatcatcatggaatacatggagaatggtgggtgctacccgagt

SEQ ID NO: 24 - DNA, 135 bp, Artificial
  ssDNA-T316M-for-sgRNA12  DNA sequence as repair template
aaaaggtgtatttccaccctctggcagggacagcagggagagcagtatcccctggtagccgactcgggtagcacccaccattctccatgtattccatgatgatgtagatgggctcctgggtgaccacagcgtaga

SEQ ID NO: 25 - DNA, 135 bp, Artificial
  ssDNA-T316A-for-sgRNA8  DNA sequence as repair template
acgccttcctggccgaggccaacctcatgaagcagctgcaacaccagcggctggttcggctctacgctgtggtcacccaggagcccatctacatcatcgccgaatacatggagaatggtgggtgctacccgagtc

SEQ ID NO: 26 - DNA, 135 bp, Artificial
  ssDNA-T316A-for-sgRNA9  DNA sequence as repair template
gacgccttcctggccgaggccaacctcatgaagcagctgcaacaccagcggctggttcggctctacgctgtggtcacccaggagcccatctacatcatcgccgaatacatggagaatggtgggtgctacccgagt

SEQ ID NO: 27 - DNA, 135 bp, Artificial
  ssDNA-T316A-for-sgRNA12  DNA sequence as repair template
aaaaggtgtatttccaccctctggcagggacagcagggagagcagtatcccctggtagccgactcgggtagcacccaccattctccatgtattccgggatgatgtagatgggctcctgggtgaccacagcgtaga

SEQ ID NO: 28 - DNA, 265 bp, Artificial
  ssDNA-T316I-for-sgRNA1+sgRNA11  DNA sequence as repair template
aggaaagctcaagaaaccctccttgcttgagctttgggccagaagaaaaggtgtatttccaccctctggcagggacagcagggagagcagtatcccctggtagccgactcgggtagcacccaccattctccatgtattcaatgatgatgtagatgggctcctgggtgaccacagcgtagagccgaaccagccgctggtgttgcagctgcttcatgaggttggcctcggccaggaaggcgtccggggacatgctgccctgcttcag

SEQ ID NO: 29 - DNA, 265 bp, Artificial
  ssDNA-T316M-for-sgRNA1+sgRNA11  DNA sequence as repair template
aggaaagctcaagaaaccctccttgcttgagctttgggccagaagaaaaggtgtatttccaccctctggcagggacagcagggagagcagtatcccctggtagccgactcgggtagcacccaccattctccatgtattccatgatgatgtagatgggctcctgggtgaccacagcgtagagccgaaccagccgctggtgttgcagctgcttcatgaggttggcctcggccaggaaggcgtccggggacatgctgccctgcttcag

SEQ ID NO: 30 - DNA, 265 bp, Artificial
  ssDNA-T316A-for-sgRNA1+sgRNA11  DNA sequence as repair template
aggaaagctcaagaaaccctccttgcttgagctttgggccagaagaaaaggtgtatttccaccctctggcagggacagcagggagagcagtatcccctggtagccgactcgggtagcacccaccattctccatgtattccgggatgatgtagatgggctcctgggtgaccacagcgtagagccgaaccagccgctggtgttgcagctgcttcatgaggttggcctcggccaggaaggcgtccggggacatgctgccctgcttcag

SEQ ID NO: 31 - DNA, 235 bp, Artificial
  ssDNA-T316I-for-sgRNA1+sgRNA12  DNA sequence as repair template
aggaaagctcaagaaaccctccttgcttgagctttgggccagaagaaaaggtgtatttccaccctctggcagggacagcagggagagcagtatcccctggtagccgactcgggtagcacccaccattctccatgtattcaatgatgatgtagatgggctcctgggtgaccacagcgtagagccgaaccagccgctggtgttgcagctgcttcatgaggttggcctcggccaggaa

SEQ ID NO: 32 - DNA, 235 bp, Artificial
  ssDNA-T316M-for-sgRNA1+sgRNA12  DNA sequence as repair template
aggaaagctcaagaaaccctccttgcttgagctttgggccagaagaaaaggtgtatttccaccctctggcagggacagcagggagagcagtatcccctggtagccgactcgggtagcacccaccattctccatgtattccatgatgatgtagatgggctcctgggtgaccacagcgtagagccgaaccagccgctggtgttgcagctgcttcatgaggttggcctcggccaggaa

SEQ ID NO: 33 - DNA, 235 bp, Artificial
  ssDNA-T316A-for-sgRNA1+sgRNA12  DNA sequence as repair template
aggaaagctcaagaaaccctccttgcttgagctttgggccagaagaaaaggtgtatttccaccctctggcagggacagcagggagagcagtatcccctggtagccgactcgggtagcacccaccattctccatgtattccgggatgatgtagatgggctcctgggtgaccacagcgtagagccgaaccagccgctggtgttgcagctgcttcatgaggttggcctcggccaggaa

SEQ ID NO: 34 - protein, 1690 aa, Escherichia coli
MEASPASGPRHLMDPHIFTSNFNNGIGRHKTYLCYEVERLDNGTSVKMDQHRGFLHNQAKNLLCGFYGRHAELRFLDLVPSLQLDPAQIYRVTWFISWSPCFSWGCAGEVRAFLQENTHVRLRIFAARIYDYDPLYKEALQMLRDAGAQVSIMTYDEFKHCWDTFVDHQGCPFQPWDGLDEHSQALSGRLRAILQNQGNSGSETPGTSESATPESDKKYSIGLAIGTNSVGWAVITDEYKVPSKKFKVLGNTDRHSIKKNLIGALLFDSGETAEATRLKRTARRRYTRRKNRICYLQEIFSNEMAKVDDSFFHRLEESFLVEEDKKHERHPIFGNIVDEVAYHEKYPTIYHLRKKLVDSTDKADLRLIYLALAHMIKFRGHFLIEGDLNPDNSDVDKLFIQLVQTYNQLFEENPINASGVDAKAILSARLSKSRRLENLIAQLPGEKKNGLFGNLIALSLGLTPNFKSNFDLAEDAKLQLSKDTYDDDLDNLLAQIGDQYADLFLAAKNLSDAILLSDILRVNTEITKAPLSASMIKRYDEHHQDLTLLKALVRQQLPEKYKEIFFDQSKNGYAGYIDGGASQEEFYKFIKPILEKMDGTEELLVKLNREDLLRKQRTFDNGSIPHQIHLGELHAILRRQEDFYPFLKDNREKIEKILTFRIPYYVGPLARGNSRFAWMTRKSEETITPWNFEEVVDKGASAQSFIERMTNFDKNLPNEKVLPKHSLLYEYFTVYNELTKVKYVTEGMRKPAFLSGEQKKAIVDLLFKTNRKVTVKQLKEDYFKKIECFDSVEISGVEDRFNASLGTYHDLLKIIKDKDFLDNEENEDILEDIVLTLTLFEDREMIEERLKTYAHLFDDKVMKQLKRRRYTGWGRLSRKLINGIRDKQSGKTILDFLKSDGFANRNFMQLIHDDSLTFKEDIQKAQVSGQGDSLHEHIANLAGSPAIKKGILQTVKVVDELVKVMGRHKPENIVIEMARENQTTQKGQKNSRERMKRIEEGIKELGSQILKEHPVENTQLQNEKLYLYYLQNGRDMYVDQELDINRLSDYDVDHIVPQSFLKDDSIDNKVLTRSDKNRGKSDNVPSEEVVKKMKNYWRQLLNAKLITQRKFDNLTKAERGGLSELDKAGFIKRQLVETRQITKHVAQILDSRMNTKYDENDKLIREVKVITLKSKLVSDFRKDFQFYKVREINNYHHAHDAYLNAVVGTALIKKYPKLESEFVYGDYKVYDVRKMIAKSEQEIGKATAKYFFYSNIMNFFKTEITLANGEIRKRPLIETNGETGEIVWDKGRDFATVRKVLSMPQVNIVKKTEVQTGGFSKESILPKRNSDKLIARKKDWDPKKYGGFDSPTVAYSVLVVAKVEKGKSKKLKSVKELLGITIMERSSFEKNPIDFLEAKGYKEVKKDLIIKLPKYSLFELENGRKRMLASAGELQKGNELALPSKYVNFLYLASHYEKLKGSPEDNEQKQLFVEQHKHYLDEIIEQISEFSKRVILADANLDKVLSAYNKHRDKPIREQAENIIHLFTLTNLGAPAAFKYFDTTIDRKRYTSTKEVLDATLIHQSITGLYETRIDLSQLGGDSGGSTNLSDIIEKETGKQLVIQESILMLPEEVEEVIGNKPESDILVHTAYDESTDENVMLLTSDAPEYKPWALVIQDSNGENKIKMLSGGSPKKKRKVHHHHHHHHHH

SEQ ID NO: 35 - DNA, 333 bp, Artificial
  CD19-78 VL nucleic acid sequence
caggctgtgctgactcagccaccctcggtgtctgaagcccccaggcagagggtcaccatctcctgttctggaagcagctccaacatcggaaataatgctgtaagctggtaccagcagctcccaggaaaggctcccaaactcctcatctattatgatgatctgctcccctcaggggtctctgaccgattctctggctccaagtctggcacctcagcctccctggccatcagtgggctccagtctgaggatgaggctgattattactgtgcagcatgggatgacagcctgaatggttgggtgttcggcggagggaccaaggtcaccgtcctaggt

SEQ ID NO: 36 - protein, 111 aa, Artificial
  CD19-78 VL protein sequence
QAVLTQPPSVSEAPRQRVTISCSGSSSNIGNNAVSWYQQLPGKAPKLLIYYDDLLPSGVSDRFSGSKSGTSASLAISGLQSEDEADYYCAAWDDSLNGWVFGGGTKVTVLG

SEQ ID NO: 37 - DNA, 363 bp, Artificial
  CD19-78 VH nucleic acid sequence
gaggtgcagctggtgcagtctggagcagaggtgaaaaagcccggggagtctctgaagatctcctgtaagggttctggatacagctttaccagctactggatcggctgggtgcgccagatgcccgggaaaggcctggagtggatggggatcatctatcctggtgactctgataccagatacagcccgtccttccaaggccaggtcaccatctcagccgacaagtccatcagcaccgcctacctgcagtggagcagcctgaaggcctcggacaccgccatgtattactgtgcgcgcctgtcttactcttggtcttcttggtactgggatttctggggtcaaggtactctggtgaccgtctcctca

SEQ ID NO: 38 - protein, 121 aa, Artificial
  CD19-78 VH protein sequence
EVQLVQSGAEVKKPGESLKISCKGSGYSFTSYWIGWVRQMPGKGLEWMGIIYPGDSDTRYSPSFQGQVTISADKSISTAYLQWSSLKASDTAMYYCARLSYSWSSWYWDFWGQGTLVTVSS

SEQ ID NO: 39 - DNA, 45 bp, Artificial
  CD19-Linker1  nucleic acid sequence
ggtggtggtggtagcggcggcggcggctctggtggtggtggatcc

SEQ ID NO: 40 - protein, 15 aa, Artificial
  CD19-Linker1  protein sequence
GGGGSGGGGSGGGGS

SEQ ID NO: 41 - DNA, 135 bp, Artificial
  CD19-CD8a hinge nucleic acid sequence
actactacccctgcacctaggcctcccaccccagccccaacaatcgccagccagcctctgtctctgcggcccgaagcctgtagacctgctgccggcggagccgtgcacaccagaggcctggacttcgcctgcgac

SEQ ID NO: 42 - protein, 45 aa, Artificial
  CD19-CD8a hinge protein sequence
TTTPAPRPPTPAPTIASQPLSLRPEACRPAAGGAVHTRGLDFACD

SEQ ID NO: 43 - DNA, 72 bp, Artificial
  CD19-CD8a TM nucleic acid sequence
atctacatctgggcccctctggccggcacctgtggcgtgctgctgctgagcctggtgatcaccctgtactgc

SEQ ID NO: 44 - protein, 24 aa, Artificial
  CD19-CD8a TM protein sequence
IYIWAPLAGTCGVLLLSLVITLYC

SEQ ID NO: 45 - DNA, 123 bp, Artificial
  CD19-CD28 intracellular domain (IC) nucleic acid sequence
agaagcaagcggagccggctgctgcacagcgactacatgaacatgaccccaagacggcctggccccacccggaagcactaccagccttacgcccctcccagagacttcgccgcctaccggtcc

SEQ ID NO: 46 - protein, 41 aa, Artificial
  CD19-CD28 intracellular domain (IC) protein sequence
RSKRSRLLHSDYMNMTPRRPGPTRKHYQPYAPPRDFAAYRS

SEQ ID NO: 47 - DNA, 336 bp, Artificial
  CD19-CD3z intracellular signaling domain nucleic acid sequence
agagtgaagttcagcagatccgccgacgcccctgcctaccagcagggacagaaccagctgtacaacgagctgaacctgggcagacgggaagagtacgacgtgctggacaagcggagaggccgggaccccgagatgggcggaaagcccagacggaagaacccccaggaaggcctgtataacgaactgcagaaagacaagatggccgaggcctacagcgagatcggcatgaagggcgagcggaggcgcggcaagggccacgatggcctgtaccagggcctgagcaccgccaccaaggacacctacgacgccctgcacatgcaggccctgccccccaga

SEQ ID NO: 48 - protein, 112 aa, Artificial
  CD19-CD3z intracellular signaling domain protein sequence
RVKFSRSADAPAYQQGQNQLYNELNLGRREEYDVLDKRRGRDPEMGGKPRRKNPQEGLYNELQKDKMAEAYSEIGMKGERRRGKGHDGLYQGLSTATKDTYDALHMQALPPR

SEQ ID NO: 49 - DNA, 54 bp, Artificial
  CD19-T2A nucleic acid sequence
gagggaaggggcagcttattaacatgtggcgatgtggaagagaaccccggtccc

SEQ ID NO: 50 - protein, 18 aa, Artificial
  CD19-T2A protein sequence
EGRGSLLTCGDVEENPGP

SEQ ID NO: 51 - DNA, 66 bp, Artificial
  CD19-CSF2RA signal nucleic acid sequence
atgctgctgctcgtgacctctttactgttatgtgagctgccccaccccgcttttttactgatccct

SEQ ID NO: 52 - protein, 22 aa, Artificial
  CD19-CSF2RA signal protein sequence
MLLLVTSLLLCELPHPAFLLIP

SEQ ID NO: 53 - DNA, 1005 bp, Artificial
  CD19-tEGFR nucleic acid sequence
cgtaaggtgtgtaacggaatcggcattggcgagttcaaggactctttaagcatcaacgccacaaacatcaagcacttcaagaattgtacctccatcagcggcgatttacacattctccccgtggcttttcgtggcgattccttcacccacaccccccctctggacccccaagagctggacattttaaaaaccgtgaaggagatcaccggctttctgctgatccaagcttggcccgagaatcgtaccgacctccacgccttcgagaatttagagattattcgtggaaggaccaagcagcacggccagttctctttagccgtcgtgtctttaaacattaccagcctcggtttaaggtctttaaaggagattagcgacggcgacgtgatcatctccggcaacaagaacctctgctacgccaacaccatcaactggaagaagctgttcggaaccagcggccaaaagaccaagatcatcagcaatcgtggagagaactcttgtaaggccactggtcaagtttgccacgccctctgtagccccgaaggatgttggggccccgagcctagggactgtgttagctgcagaaacgtgagcagaggcagagagtgtgtggacaaatgcaatttactggaaggagagcctagggagttcgtggagaacagcgaatgtatccagtgccaccccgagtgtttacctcaagccatgaacatcacttgtaccggaaggggccccgataactgcatccaatgcgcccactacatcgacggaccccactgcgtgaaaacttgtcccgccggagtgatgggagagaataacactttagtgtggaagtacgccgacgctggccacgtctgccatctgtgccaccccaactgtacctacggctgcactggtcccggtttagagggatgtcctaccaacggccccaagatcccctccatcgccaccggaatggtgggcgctctgttattactgctggtggtggctctgggcatcggtttattcatg

SEQ ID NO: 54 - protein, 335 aa, Artificial
  CD19-tEGFR protein sequence
RKVCNGIGIGEFKDSLSINATNIKHFKNCTSISGDLHILPVAFRGDSFTHTPPLDPQELDILKTVKEITGFLLIQAWPENRTDLHAFENLEIIRGRTKQHGQFSLAVVSLNITSLGLRSLKEISDGDVIISGNKNLCYANTINWKKLFGTSGQKTKIISNRGENSCKATGQVCHALCSPEGCWGPEPRDCVSCRNVSRGRECVDKCNLLEGEPREFVENSECIQCHPECLPQAMNITCTGRGPDNCIQCAHYIDGPHCVKTCPAGVMGENNTLVWKYADAGHVCHLCHPNCTYGCTGPGLEGCPTNGPKIPSIATGMVGALLLLLVVALGIGLFM

SEQ ID NO: 55 - DNA, 2649 bp, Artificial
  CD19-CD28z-CAR nucleic acid sequence
atggccctgcctgtgacagctctgctcctccctctggccctgctgctccatgccgccagaccccaggctgtgctgactcagccaccctcggtgtctgaagcccccaggcagagggtcaccatctcctgttctggaagcagctccaacatcggaaataatgctgtaagctggtaccagcagctcccaggaaaggctcccaaactcctcatctattatgatgatctgctcccctcaggggtctctgaccgattctctggctccaagtctggcacctcagcctccctggccatcagtgggctccagtctgaggatgaggctgattattactgtgcagcatgggatgacagcctgaatggttgggtgttcggcggagggaccaaggtcaccgtcctaggtggtggtggtggtagcggcggcggcggctctggtggtggtggatccgaggtgcagctggtgcagtctggagcagaggtgaaaaagcccggggagtctctgaagatctcctgtaagggttctggatacagctttaccagctactggatcggctgggtgcgccagatgcccgggaaaggcctggagtggatggggatcatctatcctggtgactctgataccagatacagcccgtccttccaaggccaggtcaccatctcagccgacaagtccatcagcaccgcctacctgcagtggagcagcctgaaggcctcggacaccgccatgtattactgtgcgcgcctgtcttactcttggtcttcttggtactgggatttctggggtcaaggtactctggtgaccgtctcctcattcgtgcccgtgttcctgcccgccaaacctactactacccctgcacctaggcctcccaccccagccccaacaatcgccagccagcctctgtctctgcggcccgaagcctgtagacctgctgccggcggagccgtgcacaccagaggcctggacttcgcctgcgacatctacatctgggcccctctggccggcacctgtggcgtgctgctgctgagcctggtgatcaccctgtactgcaaccaccggaacagaagcaagcggagccggctgctgcacagcgactacatgaacatgaccccaagacggcctggccccacccggaagcactaccagccttacgcccctcccagagacttcgccgcctaccggtccagagtgaagttcagcagatccgccgacgcccctgcctaccagcagggacagaaccagctgtacaacgagctgaacctgggcagacgggaagagtacgacgtgctggacaagcggagaggccgggaccccgagatgggcggaaagcccagacggaagaacccccaggaaggcctgtataacgaactgcagaaagacaagatggccgaggcctacagcgagatcggcatgaagggcgagcggaggcgcggcaagggccacgatggcctgtaccagggcctgagcaccgccaccaaggacacctacgacgccctgcacatgcaggccctgccccccagaggatccggagagggaaggggcagcttattaacatgtggcgatgtggaagagaaccccggtcccatgctgctgctcgtgacctctttactgttatgtgagctgccccaccccgcttttttactgatccctcgtaaggtgtgtaacggaatcggcattggcgagttcaaggactctttaagcatcaacgccacaaacatcaagcacttcaagaattgtacctccatcagcggcgatttacacattctccccgtggcttttcgtggcgattccttcacccacaccccccctctggacccccaagagctggacattttaaaaaccgtgaaggagatcaccggctttctgctgatccaagcttggcccgagaatcgtaccgacctccacgccttcgagaatttagagattattcgtggaaggaccaagcagcacggccagttctctttagccgtcgtgtctttaaacattaccagcctcggtttaaggtctttaaaggagattagcgacggcgacgtgatcatctccggcaacaagaacctctgctacgccaacaccatcaactggaagaagctgttcggaaccagcggccaaaagaccaagatcatcagcaatcgtggagagaactcttgtaaggccactggtcaagtttgccacgccctctgtagccccgaaggatgttggggccccgagcctagggactgtgttagctgcagaaacgtgagcagaggcagagagtgtgtggacaaatgcaatttactggaaggagagcctagggagttcgtggagaacagcgaatgtatccagtgccaccccgagtgtttacctcaagccatgaacatcacttgtaccggaaggggccccgataactgcatccaatgcgcccactacatcgacggaccccactgcgtgaaaacttgtcccgccggagtgatgggagagaataacactttagtgtggaagtacgccgacgctggccacgtctgccatctgtgccaccccaactgtacctacggctgcactggtcccggtttagagggatgtcctaccaacggccccaagatcccctccatcgccaccggaatggtgggcgctctgttattactgctggtggtggctctgggcatcggtttattcatgtga

SEQ ID NO: 56 - protein, 882 aa, Artificial
  CD19-CD28z-CAR protein sequence
MALPVTALLLPLALLLHAARPQAVLTQPPSVSEAPRQRVTISCSGSSSNIGNNAVSWYQQLPGKAPKLLIYYDDLLPSGVSDRFSGSKSGTSASLAISGLQSEDEADYYCAAWDDSLNGWVFGGGTKVTVLGGGGGSGGGGSGGGGSEVQLVQSGAEVKKPGESLKISCKGSGYSFTSYWIGWVRQMPGKGLEWMGIIYPGDSDTRYSPSFQGQVTISADKSISTAYLQWSSLKASDTAMYYCARLSYSWSSWYWDFWGQGTLVTVSSFVPVFLPAKPTTTPAPRPPTPAPTIASQPLSLRPEACRPAAGGAVHTRGLDFACDIYIWAPLAGTCGVLLLSLVITLYCNHRNRSKRSRLLHSDYMNMTPRRPGPTRKHYQPYAPPRDFAAYRSRVKFSRSADAPAYQQGQNQLYNELNLGRREEYDVLDKRRGRDPEMGGKPRRKNPQEGLYNELQKDKMAEAYSEIGMKGERRRGKGHDGLYQGLSTATKDTYDALHMQALPPRGSGEGRGSLLTCGDVEENPGPMLLLVTSLLLCELPHPAFLLIPRKVCNGIGIGEFKDSLSINATNIKHFKNCTSISGDLHILPVAFRGDSFTHTPPLDPQELDILKTVKEITGFLLIQAWPENRTDLHAFENLEIIRGRTKQHGQFSLAVVSLNITSLGLRSLKEISDGDVIISGNKNLCYANTINWKKLFGTSGQKTKIISNRGENSCKATGQVCHALCSPEGCWGPEPRDCVSCRNVSRGRECVDKCNLLEGEPREFVENSECIQCHPECLPQAMNITCTGRGPDNCIQCAHYIDGPHCVKTCPAGVMGENNTLVWKYADAGHVCHLCHPNCTYGCTGPGLEGCPTNGPKIPSIATGMVGALLLLLVVALGIGLFM

SEQ ID NO: 57 - DNA, 354 bp, Artificial
  CD5-Ab20001-61-VH nucleic acid sequence
caggtgcagctggtgcagtctggggctgaggtgaagaagcctgggtcctcggtgaaggtctcctgcaaggcttctggaggcaccttcagcaactatgctatcagctgggtgcgacaggcccctggacaagggcttgagtggatgggatggatcagcgcctacaatggtgacacaaaatatgcacagaggctccagggcagagtcaccatgaccacagacacatccacgagcacagcctacatggagctgaggaacctaagatctgacgacacggccgtgtattactgtgcgcgctacgaatctatgtctggtcaggatatctggggtcaaggtactctggtgaccgtctcctca

SEQ ID NO: 58 - protein, 118 aa, Artificial
  CD5-Ab20001-61-VH protein sequence
QVQLVQSGAEVKKPGSSVKVSCKASGGTFSNYAISWVRQAPGQGLEWMGWISAYNGDTKYAQRLQGRVTMTTDTSTSTAYMELRNLRSDDTAVYYCARYESMSGQDIWGQGTLVTVSS

SEQ ID NO: 59 - DNA, 363 bp, Artificial
  CD5-Ab20001-42-VH nucleic acid sequence
gaagttcagctgctggaaagcggtggtggtctggttcagcctggtggtagcctgcgtctgagctgtgcagcaagcggttttacctttagccatagcgccatgggttgggttcgtcaggcacctggtaaaggtctggaatgggttagcagcatctatgcccgcggcggctatacctattatgcagatagcgttaaaggtcgttttaccattagccgtgataacagcaaaaataccctgtacctgcagatgaatagtctgcgtgcagaggataccgcagtgtattattgtgcgcgcggttaccatctggaatacatggtttctcaggatgtttggggtcaaggtactctggtgaccgtctcctca

SEQ ID NO: 60 - protein, 121 aa, Artificial
  CD5-Ab20001-42-VH protein sequence
EVQLLESGGGLVQPGGSLRLSCAASGFTFSHSAMGWVRQAPGKGLEWVSSIYARGGYTYYADSVKGRFTISRDNSKNTLYLQMNSLRAEDTAVYYCARGYHLEYMVSQDVWGQGTLVTVSS

SEQ ID NO: 61 - DNA, 45 bp, Artificial; identical to SEQ ID NO: 39
  CD5-Linker1  nucleic acid sequence

SEQ ID NO: 62 - protein, 15 aa, Artificial
  CD5-Linker1  protein sequence
GGGGSGGGGSGGGGS

SEQ ID NO: 63 - DNA, 381 bp, Artificial
  CD5-CD8a nucleic acid sequence
tttgtgcctgtatttctgcctgccaagcccaccacaacacctgcccctagaccacccacccctgcccccaccattgcttctcagccccttagcttaagacctgaagcctgtagacctgctgctgggggggctgtgcacacaagaggcctggactttgcctgtactactacccctgcacctaggcctcccaccccagccccaacaatcgccagccagcctctgtctctgcggcccgaagcctgtagacctgctgccggcggagccgtgcacaccagaggcctggacttcgcctgcgacatctacatctgggcccccctggctggcacctgtggggtgctgctgctgagcctggtgatcaccctgtactgcaaccacagaaac

SEQ ID NO: 64 - protein, 127 aa, Artificial
  CD5-CD8a protein sequence
FVPVFLPAKPTTTPAPRPPTPAPTIASQPLSLRPEACRPAAGGAVHTRGLDFACTTTPAPRPPTPAPTIASQPLSLRPEACRPAAGGAVHTRGLDFACDIYIWAPLAGTCGVLLLSLVITLYCNHRN

SEQ ID NO: 65 - DNA, 123 bp, Artificial
  CD5-CD28 intracellular domain (IC) nucleic acid sequence
aggagtaagaggagcaggctcctgcacagtgactacatgaacatgactccccgccgccccgggcccacccgcaagcattaccagccctatgccccaccacgcgacttcgcagcctatcgctcc

SEQ ID NO: 66 - protein, 41 aa, Artificial; identical to SEQ ID NO: 46
  CD5-CD28 intracellular domain (IC) protein sequence

SEQ ID NO: 67 - DNA, 336 bp, Artificial
  CD5-CD3z intracellular signaling domain nucleic acid sequence
agagtgaagttcagcagatctgctgatgcccctgcctatcagcaagggcagaatcagctgtacaatgagctgaatctgggcagaagagaggagtatgatgtgctggacaagagaagaggcagagaccctgagatggggggcaagcctagaagaaagaacccccaagagggcctgtataatgagctgcagaaggacaagatggctgaggcctactctgagattggcatgaagggggagagaagaagaggcaagggccatgatggcctgtaccaaggcctgagcacagccaccaaggacacctatgatgccctacacatgcaagctctgcctcctaga

SEQ ID NO: 68 - protein, 112 aa, Artificial; identical to SEQ ID NO: 48
  CD5-CD3z intracellular signaling domain protein sequence

SEQ ID NO: 69 - DNA, 54 bp, Artificial
  CD5-T2A nucleic acid sequence
gaaggaaggggcagcctactgacctgtggggatgtggaggagaaccctggcccc

SEQ ID NO: 70 - protein, 18 aa, Artificial
  CD5-T2A protein sequence
EGRGSLLTCGDVEENPGP

SEQ ID NO: 71 - DNA, 66 bp, Artificial
  CD5-CSF2RA signal nucleic acid sequence
atgttgctattagtaaccagcctgctgctgtgtgagctgccccaccctgccttcctgttaatccca

SEQ ID NO: 72 - protein, 22 aa, Artificial
  CD5-CSF2RA signal protein sequence
MLLLVTSLLLCELPHPAFLLIP

SEQ ID NO: 73 - DNA, 1005 bp, Artificial
  CD5-tEGFR nucleic acid sequence
cgaaaggtatgtaatggcattggcattggggagtttaaggacagcctgagcatcaatgccaccaacatcaagcacttcaagaactgcacaagcatcagtggggacttgcacatcctgcctgtggccttcagaggggacagcttcacccacaccccccccctggacccccaagagctggacatcctgaagacagtgaaggagatcactggcttcttgctgatccaagcctggcctgagaacagaacagacctgcatgcctttgagaacctggagatcatcagaggcagaaccaagcagcatgggcagttcagcctggctgtggtgagcctgaacatcacaagcctgggcctgagaagcttaaaggagatctctgatggggatgtgatcatctctggcaacaagaacctgtgctatgccaacaccatcaactggaagaagctgtttggcacctctgggcagaagaccaagatcatcagcaacagaggggagaactcctgtaaggccactggccaagtgtgtcatgccctatgcagccctgaggggtgctggggccctgagcctagagactgtgtgagctgcagaaatgtgagcagaggcagagagtgtgtggacaagtgcaacctgctggagggggagcctagagagtttgtggagaactctgagtgtattcagtgtcatcctgagtgcctgccccaagccatgaacatcacctgcactggcagaggccctgacaactgcattcagtgtgcccactacattgatggcccccactgtgtgaagacctgccctgctggggtgatgggggagaacaacaccctggtgtggaagtatgctgatgctggccatgtgtgtcacctgtgccatcccaactgcacctatggctgcactggccctggcctggagggctgccccaccaatggtcccaagattcctagcattgccactggcatggtgggggccctgctcctacttctggtggttgccctgggcattggcctgttcatg

SEQ ID NO: 74 - protein, 335 aa, Artificial; identical to SEQ ID NO: 54
  CD5-tEGFR protein sequence

SEQ ID NO: 75 - DNA, 2670 bp, Artificial
  CD5-VHH-CD28z-CAR nucleic acid sequence
atggccctacctgtgacagccctactgttacccctggccctccttctgcatgctgctagacctcaggtgcagctggtgcagtctggggctgaggtgaagaagcctgggtcctcggtgaaggtctcctgcaaggcttctggaggcaccttcagcaactatgctatcagctgggtgcgacaggcccctggacaagggcttgagtggatgggatggatcagcgcctacaatggtgacacaaaatatgcacagaggctccagggcagagtcaccatgaccacagacacatccacgagcacagcctacatggagctgaggaacctaagatctgacgacacggccgtgtattactgtgcgcgctacgaatctatgtctggtcaggatatctggggtcaaggtactctggtgaccgtctcctcagggggggggggctctggggggggtggctcaggtggcggtggctctgaagttcagctgctggaaagcggtggtggtctggttcagcctggtggtagcctgcgtctgagctgtgcagcaagcggttttacctttagccatagcgccatgggttgggttcgtcaggcacctggtaaaggtctggaatgggttagcagcatctatgcccgcggcggctatacctattatgcagatagcgttaaaggtcgttttaccattagccgtgataacagcaaaaataccctgtacctgcagatgaatagtctgcgtgcagaggataccgcagtgtattattgtgcgcgcggttaccatctggaatacatggtttctcaggatgtttggggtcaaggtactctggtgaccgtctcctcatttgtgcctgtatttctgcctgccaagcccaccacaacacctgcccctagaccacccacccctgcccccaccattgcttctcagccccttagcttaagacctgaagcctgtagacctgctgctgggggggctgtgcacacaagaggcctggactttgcctgtgacatctacatctgggcccccctggctggcacctgtggggtgctgctgctgagcctggtgatcaccctgtactgcaaccacagaaacaggagtaagaggagcaggctcctgcacagtgactacatgaacatgactccccgccgccccgggcccacccgcaagcattaccagccctatgccccaccacgcgacttcgcagcctatcgctccagagtgaagttcagcagatctgctgatgcccctgcctatcagcaagggcagaatcagctgtacaatgagctgaatctgggcagaagagaggagtatgatgtgctggacaagagaagaggcagagaccctgagatggggggcaagcctagaagaaagaacccccaagagggcctgtataatgagctgcagaaggacaagatggctgaggcctactctgagattggcatgaagggggagagaagaagaggcaagggccatgatggcctgtaccaaggcctgagcacagccaccaaggacacctatgatgccctacacatgcaagctctgcctcctagaggctctggggaaggaaggggcagcctactgacctgtggggatgtggaggagaaccctggccccatgttgctattagtaaccagcctgctgctgtgtgagctgccccaccctgccttcctgttaatcccacgaaaggtatgtaatggcattggcattggggagtttaaggacagcctgagcatcaatgccaccaacatcaagcacttcaagaactgcacaagcatcagtggggacttgcacatcctgcctgtggccttcagaggggacagcttcacccacaccccccccctggacccccaagagctggacatcctgaagacagtgaaggagatcactggcttcttgctgatccaagcctggcctgagaacagaacagacctgcatgcctttgagaacctggagatcatcagaggcagaaccaagcagcatgggcagttcagcctggctgtggtgagcctgaacatcacaagcctgggcctgagaagcttaaaggagatctctgatggggatgtgatcatctctggcaacaagaacctgtgctatgccaacaccatcaactggaagaagctgtttggcacctctgggcagaagaccaagatcatcagcaacagaggggagaactcctgtaaggccactggccaagtgtgtcatgccctatgcagccctgaggggtgctggggccctgagcctagagactgtgtgagctgcagaaatgtgagcagaggcagagagtgtgtggacaagtgcaacctgctggagggggagcctagagagtttgtggagaactctgagtgtattcagtgtcatcctgagtgcctgccccaagccatgaacatcacctgcactggcagaggccctgacaactgcattcagtgtgcccactacattgatggcccccactgtgtgaagacctgccctgctggggtgatgggggagaacaacaccctggtgtggaagtatgctgatgctggccatgtgtgtcacctgtgccatcccaactgcacctatggctgcactggccctggcctggagggctgccccaccaatggtcccaagattcctagcattgccactggcatggtgggggccctgctcctacttctggtggttgccctgggcattggcctgttcatgtga

SEQ ID NO: 76 - protein, 889 aa, Artificial
  CD5-VHH-CD28z-CAR protein sequence
MALPVTALLLPLALLLHAARPQVQLVQSGAEVKKPGSSVKVSCKASGGTFSNYAISWVRQAPGQGLEWMGWISAYNGDTKYAQRLQGRVTMTTDTSTSTAYMELRNLRSDDTAVYYCARYESMSGQDIWGQGTLVTVSSGGGGSGGGGSGGGGSEVQLLESGGGLVQPGGSLRLSCAASGFTFSHSAMGWVRQAPGKGLEWVSSIYARGGYTYYADSVKGRFTISRDNSKNTLYLQMNSLRAEDTAVYYCARGYHLEYMVSQDVWGQGTLVTVSSFVPVFLPAKPTTTPAPRPPTPAPTIASQPLSLRPEACRPAAGGAVHTRGLDFACDIYIWAPLAGTCGVLLLSLVITLYCNHRNRSKRSRLLHSDYMNMTPRRPGPTRKHYQPYAPPRDFAAYRSRVKFSRSADAPAYQQGQNQLYNELNLGRREEYDVLDKRRGRDPEMGGKPRRKNPQEGLYNELQKDKMAEAYSEIGMKGERRRGKGHDGLYQGLSTATKDTYDALHMQALPPRGSGEGRGSLLTCGDVEENPGPMLLLVTSLLLCELPHPAFLLIPRKVCNGIGIGEFKDSLSINATNIKHFKNCTSISGDLHILPVAFRGDSFTHTPPLDPQELDILKTVKEITGFLLIQAWPENRTDLHAFENLEIIRGRTKQHGQFSLAVVSLNITSLGLRSLKEISDGDVIISGNKNLCYANTINWKKLFGTSGQKTKIISNRGENSCKATGQVCHALCSPEGCWGPEPRDCVSCRNVSRGRECVDKCNLLEGEPREFVENSECIQCHPECLPQAMNITCTGRGPDNCIQCAHYIDGPHCVKTCPAGVMGENNTLVWKYADAGHVCHLCHPNCTYGCTGPGLEGCPTNGPKIPSIATGMVGALLLLLVVALGIGLFM

SEQ ID NO: 77 - DNA, 1464 bp, Artificial
  BCMA-CAR nucleic acid sequence
tacccatacgatgttccagattacgctgacatccagatgacccagtctccatcctccctgtctgcatctgtaggagacagagtcaccatcacttgccgggcaagtcagagcattagcagctatttaaattggtatcagcagaaaccagggaaagcccctaagctcctgatctatgctgcatccagtttgcaaagtggggtcccatcaaggttcagtggcagtggatctgggacagatttcactctcaccatcagcagtctgcaacctgaagattttgcaacttactactgtcagcaaaaatacgacctcctcacttttggcggagggaccaaggttgagatcaaaggcagcaccagcggctccggcaagcctggctctggcgagggcagcacaaagggacagctgcagctgcaggagtcgggcccaggactggtgaagccttcggagaccctgtccctcacctgcactgtctctggtggctccatcagcagtagtagttactactggggctggatccgccagcccccagggaaggggctggagtggattgggagtatctcctatagtgggagcacctactacaacccgtccctcaagagtcgagtcaccatatccgtagacacgtccaagaaccagttctccctgaagctgagttctgtgaccgccgcagacacggcggtgtactactgcgccagagatcgtggagacaccatactagacgtatggggtcagggtacaatggtcaccgtcagctcattcgtgcccgtgttcctgcccgccaaacctaccaccacccctgcccctagacctcccaccccagccccaacaatcgccagccagcctctgtctctgcggcccgaagcctgtagacctgctgccggcggagccgtgcacaccagaggcctggacttcgcctgcgacatctacatctgggcccctctggccggcacctgtggcgtgctgctgctgagcctggtgatcaccctgtactgcaaccaccggaacagaagcaagcggagccggctgctgcacagcgactacatgaacatgaccccaagacggcctggccccacccggaagcactaccagccttacgcccctcccagagacttcgccgcctaccggtccagagtgaagttcagcagatccgccgacgcccctgcctaccagcagggacagaaccagctgtacaacgagctgaacctgggcagacgggaagagtacgacgtgctggacaagcggagaggccgggaccccgagatgggcggaaagcccagacggaagaacccccaggaaggcctgtataacgaactgcagaaagacaagatggccgaggcctacagcgagatcggcatgaagggcgagcggaggcgcggcaagggccacgatggcctgtaccagggcctgagcaccgccaccaaggacacctacgacgccctgcacatgcaggccctgccccccaga

SEQ ID NO: 78 - protein, 488 aa, Artificial
  BCMA-CAR protein sequence
YPYDVPDYADIQMTQSPSSLSASVGDRVTITCRASQSISSYLNWYQQKPGKAPKLLIYAASSLQSGVPSRFSGSGSGTDFTLTISSLQPEDFATYYCQQKYDLLTFGGGTKVEIKGSTSGSGKPGSGEGSTKGQLQLQESGPGLVKPSETLSLTCTVSGGSISSSSYYWGWIRQPPGKGLEWIGSISYSGSTYYNPSLKSRVTISVDTSKNQFSLKLSSVTAADTAVYYCARDRGDTILDVWGQGTMVTVSSFVPVFLPAKPTTTPAPRPPTPAPTIASQPLSLRPEACRPAAGGAVHTRGLDFACDIYIWAPLAGTCGVLLLSLVITLYCNHRNRSKRSRLLHSDYMNMTPRRPGPTRKHYQPYAPPRDFAAYRSRVKFSRSADAPAYQQGQNQLYNELNLGRREEYDVLDKRRGRDPEMGGKPRRKNPQEGLYNELQKDKMAEAYSEIGMKGERRRGKGHDGLYQGLSTATKDTYDALHMQALPPR

SEQ ID NO: 79 - protein, 177 aa, Artificial
  hIL7 amino acid sequence
MFHVSFRYIFGLPPLILVLLPVASSDCDIEGKDGKQYESVLMVSIDQLLDSMKEIGSNCLNNEFNFFKRHICDANKEGMFLFRAARKLRQFLKMNSTGDFDLHLLKVSEGTTILLNCTGQVKGRKPAALGEAQPTKSLEENKSLKEQKKLNDLCFLKRLLQEIKTCWNKILMGTKEH

SEQ ID NO: 80 - protein, 98 aa, Artificial
  CCL19 amino acid sequence
MALLLALSLLVLWTSPAPTLSGTNDAEDCCLSVTQKPIPGYIVRNFHYLLIKDGCRVPAVVFTTLRGRQLCAPPDQPWVERIIQRLQRTSAKMKRRSS

SEQ ID NO: 81 - protein, 206 aa, Artificial
  IL2RB-CD3z amino acid sequence
NCRNTGPWLKKVLKCNTPDPSKFFSQLSSEHGGDVQKWLSSPFPSSSFSPGGLAPEISPLEVLERDKVTQLLPLNTDAYLSLQELQGQDPTHLVRVKFSRSADAPAYQQGQNQLYNELNLGRREEYDVLDKRRGRDPEMGGKPRRKNPQEGLYNELQKDKMAEAYSEIGMKGERRRGKGHDGLYQGLSTATKDTYDAYRHQALPPR

SEQ ID NO: 82 - protein, 462 aa, Artificial
  IL7RaMut amino acid sequence
MTILGTTFGMVFSLLQVVSGESGYAQNGDLEDAELDDYSFSCYSQLEVNGSQHSLTCAFEDPDVNITNLEFEICGALVEVKCLNFRKLQEIYFIETKKFLLIGKSNICVKVGEKSLTCKKIDLTTIVKPEAPFDLSVVYREGANDFVVTFNTSHLQKKYVKVLMHDVAYRQEKDENKWTHVNLSSTKLTLLQRKLQPAAMYEIKVRSIPDHYFKGFWSEWSPSYYFRTPEINNSSGEMDPILLTCPTISILSFFSVALLVILACVLWKKRIKPIVWPSLPDHKKTLEHLCKKPRKNLNVSFNPESFLDCQIHRVDDIQARDEVEGFLQDTFPQQLEESEKQRLGGDVQSPNCPSEDVVITPESFGRDSSLTCLAGNVSACDAPILSSSRSLDCRESGKNGPHVYQDLLLSLGTTNSTLPPPFSLQSGILTLNPVAQGQPILTSLGSNQEEAYVTMSSFYQNQ